European Patent Application EP 4 534 107 A2, published April 9, 2025. Title: PROTEIN COMPLEX BY USE OF A SPECIFIC SITE OF AN IMMUNOGLOBULIN FRAGMENT FOR LINKAGE. Applicant: HANMI PHARM. CO., LTD. Application EP 24218489.3, filed September 26, 2016. The sequence listing filed with the application follows.

SEQUENCE LISTING (1 sequence)

SEQ ID NO: 1 - protein, 221 aa, synthetic construct
  REGION 1..221: note = human immunoclobulin Fc region derivative monomer
PSCPAPEFLGGPSVFLFPPKPKDTLMISRTPEVTCVVVDVSQEDPEVQFNWYVDGVEVHNAKTKPREEQFNSTYRVVSVLTVLHQDWLNGKEYKCKVSNKGLPSSIEKTISKAKGQPREPQVYTLPPSQEEMTKNQVSLTCLVKGFYPSDIAVEWESNGQPENNYKTTPPVLDSDGSFFLYSRLTVDKSRWQEGNVFSCSVMHEALHNHYTQKSLSLSLGK